European Patent Application EP 4 806 906 A1, published September 16, 2026. Title: VIRUS-LIKE STRUCTURED NANO-CONNECTOR AND USE THEREOF. Applicant: Eye Hospital of Shandong First Medical University (Shandong Eye Hospital). Application CN. The sequence listing filed with the application follows.

SEQUENCE LISTING (3 sequences)

SEQ ID NO: 1 - protein, 9 aa, synthetic construct
LRELHLNNN

SEQ ID NO: 2 - protein, 203 aa, synthetic construct
MDIDHYKEFGASVELLSFLPSDFFPSIRDLLDTASALYREALESPEHCSPHHTALRQAILCWGELMNLATWVGSNLEDGTSGSSGSGSGGSGSGGLRELHLNNNGSGSGGSGSGSSGSTGSRELVVGYVNVNMGLKIRQILWFHISCLTFGRETVLEYLVSFGVWIRTPPAYRPPNAPILSTLPGSGGLRELHLNNNHHHHHH

SEQ ID NO: 3 - DNA, 609 bp, synthetic construct
  source 1..609: mol_type = other DNA
atggacatcgaccattataaagagttcggcgcgagcgtggaattgctgtcgttcctgccgagcgactttttcccgagcattcgtgatctgctggataccgcttctgcactctaccgcgaggccttggagagcccggaacattgcagcccgcatcacaccgcactgcgtcaggcgattctgtgttggggtgaattaatgaacctcgctacctgggtgggttccaacttggaggacggcacgtctggctcatctggttcaggctctggtggttcaggtagtggtggcttgcgtgaactgcacctgaacaacaacggctcaggctcaggtggcagcggtagtggtagcagcggcagtacgggtagccgtgaacttgtagttggttatgttaatgttaacatgggtctgaagatccgccaaatcttatggtttcatatcagctgcctgacgtttggccgtgagacagttttggaatacctggtctccttcggggtgtggattcgtaccccgccggcgtatcgccctccgaatgccccaattctgtccaccctgccgggtagtggtggcttgcgtgaactgcacctgaacaacaaccaccaccaccaccaccac